European Patent Application EP 4 428 155 A1, published September 11, 2024. Title: ANTIBODY BINDING TO C-MET AND USE THEREOF. Applicant: Chia Tai Tianqing Pharmaceutical Group Co., Ltd. The sequence listing filed with the application follows.

SEQUENCE LISTING (47 sequences)

SEQ ID NO: 1 - DNA, 23 bp, synthetic construct
  source 1..23: mol_type = other DNA
  gene 1..23: note = Call001
gtcctggctgctcttctacaagg

SEQ ID NO: 2 - DNA, 23 bp, synthetic construct
  source 1..23: mol_type = other DNA
  gene 1..23: note = Call002
ggtacgtgctgttgaactgttcc

SEQ ID NO: 3 - DNA, 29 bp, synthetic construct
  source 1..29: mol_type = other DNA
  gene 1..29: note = V-Back
gatgtgcagctgcaggagtctggrggagg

SEQ ID NO: 4 - DNA, 34 bp, synthetic construct
  source 1..34: mol_type = other DNA
  gene 1..34: note = V-Fwd
ctagtgcggccgctgaggagacggtgacctgggt

SEQ ID NO: 5 - skipped

SEQ ID NO: 6 - protein, 17 aa, synthetic construct
  REGION 1..17: note = 1B-3B11 CDR2
VINPGGDNTDYTYAVKG

SEQ ID NO: 7 - protein, 16 aa, synthetic construct
  REGION 1..16: note = 1B-3B11 CDR3
GRTFGGTWMDRNKWKY

SEQ ID NO: 8 - protein, 5 aa, synthetic construct
  REGION 1..5: note = 1B-1B6 CDR1
SGCMG

SEQ ID NO: 9 - protein, 17 aa, synthetic construct
  REGION 1..17: note = 1B-1B6 CDR2
TIYTRNDFTYYSDSVKG

SEQ ID NO: 10 - protein, 22 aa, synthetic construct
  REGION 1..22: note = 1B-B6 CDR3
GSPFRYAGAWNVCGLKEEDYNY

SEQ ID NO: 11 - protein, 5 aa, synthetic construct
  REGION 1..5: note = 1B-1C7 CDR1
ANCVG

SEQ ID NO: 12 - protein, 17 aa, synthetic construct
  REGION 1..17: note = 1B-1C7 CDR2
AINTGGETATYADFVKG

SEQ ID NO: 13 - protein, 19 aa, synthetic construct
  REGION 1..19: note = 1B-1C7 CDR3
VGTRKYWDECSLSQHAYKN

SEQ ID NO: 14 - protein, 5 aa, synthetic construct
  REGION 1..5: note = 1B-1A8 CDR1
SYAMD

SEQ ID NO: 15 - protein, 16 aa, synthetic construct
  REGION 1..16: note = 1B-1A8 CDR2
GINSAGSPSYEASVKG

SEQ ID NO: 16 - protein, 10 aa, synthetic construct
  REGION 1..10: note = 1B-1A8 CDR3
CRDFRSPYCR

SEQ ID NO: 17 - skipped

SEQ ID NO: 18 - protein, 16 aa, synthetic construct
  REGION 1..16: note = 1B-1B2 CDR2
SISSDGNSDYLDSVKG

SEQ ID NO: 19 - protein, 19 aa, synthetic construct
  REGION 1..19: note = 1B-1B2 CDR3
NGAGHLVLRPLCGSNAVDA

SEQ ID NO: 20 - protein, 5 aa, synthetic construct
  REGION 1..5: note = 3B-1C7 CDR1
GTTMG

SEQ ID NO: 21 - protein, 16 aa, synthetic construct
  REGION 1..16: note = 3B-1C7 CDR2
DISSDGNTYYSDSVKG

SEQ ID NO: 22 - protein, 18 aa, synthetic construct
  REGION 1..18: note = 3B-1C7 CDR3
AEFRLLLRPLCRQDDYGY

SEQ ID NO: 23 - DNA, 369 bp, synthetic construct
  source 1..369: mol_type = other DNA
  gene 1..369: note = nucleotide sequence of 1B-3B11 VHH
caggtgcagctggtggagtctgggggaggctcggtgcaggctggagggtctctgagactctcctgtgtagtctctggatacacctacagtagcgtggcctggttccgccaaactccagggaaggagcgcgagggggtcgctgttataaatcctggtggtgataacaccgactatacgtatgccgtgaagggccgattcaccatctcccgagacagcgccaagagcacggtgtttctgcaaatgaacaacctggaatctgaggacactgctatgtactactgtgcggcaggacggacgttcggtggcacatggatggatcggaataagtggaagtactggggccagggcaccctggtcactgtctcatca

SEQ ID NO: 24 - protein, 123 aa, synthetic construct
  REGION 1..123: note = amino acid sequence of 1B-3B11 VHH
QVQLVESGGGSVQAGGSLRLSCVVSGYTYSSVAWFRQTPGKEREGVAVINPGGDNTDYTYAVKGRFTISRDSAKSTVFLQMNNLESEDTAMYYCAAGRTFGGTWMDRNKWKYWGQGTLVTVSS

SEQ ID NO: 25 - DNA, 393 bp, synthetic construct
  source 1..393: mol_type = other DNA
  gene 1..393: note = nucleotide sequence of 1B-1B6 VHH
caggtgcagctggtggagtctgggggagactcggtgcaggctggagggtctctgagactctcctgtgcagcctctgcacacgcctatagtagcggctgcatgggctggttccgccaggctccagggaagggccgcgagggggtcgcaactatttatactcgtaatgatttcacatactattccgactccgtgaagggccgattcaccatctcccgagacgacgccaagaacacggtgtatctgcaagtgaacagcctgaaagctgaggacactgccatgtactactgtgcggcaggttcacccttccggtacgctggtgcgtggaacgtctgcggcctgaaagaagaagactataactactggggccaggggaccctggtcactgtctcatca

SEQ ID NO: 26 - protein, 131 aa, synthetic construct
  REGION 1..131: note = amino acid sequence of 1B-1B6 VHH
QVQLVESGGDSVQAGGSLRLSCAASAHAYSSGCMGWFRQAPGKGREGVATIYTRNDFTYYSDSVKGRFTISRDDAKNTVYLQVNSLKAEDTAMYYCAAGSPFRYAGAWNVCGLKEEDYNYWGQGTLVTVSS

SEQ ID NO: 27 - DNA, 384 bp, synthetic construct
  source 1..384: mol_type = other DNA
  gene 1..384: note = nucleotide sequence of 1B-1C7 VHH
caggtgcagctggtggagtctgggggaggcttggtgcagcctggggggtctctaagactctcctgtgcagcctctggatacagttacagtgctaactgcgtgggctggttctaccaggccccagggaaggagcgcgagggggtcgcagctatcaacactggtggtgaaacggcaacttatgccgacttcgtgaagggccgattcaccatctcccaagactacgccaagaacacggtgtatctgcaaatgaacagcctcaaatctgaggacactggcatgtactactgtgcggccgtagggacgaggaagtattgggacgagtgctccctttctcaacatgcgtataaaaactggggccagggcaccctggtcactgtctcatca

SEQ ID NO: 28 - protein, 128 aa, synthetic construct
  REGION 1..128: note = amino acid sequence of 1B-1C7 VHH
QVQLVESGGGLVQPGGSLRLSCAASGYSYSANCVGWFYQAPGKEREGVAAINTGGETATYADFVKGRFTISQDYAKNTVYLQMNSLKSEDTGMYYCAAVGTRKYWDECSLSQHAYKNWGQGTLVTVSS

SEQ ID NO: 29 - DNA, 354 bp, synthetic construct
  source 1..354: mol_type = other DNA
  gene 1..354: note = nucleotide sequence of 1B-1A8 VHH
gaggtgcagctggtggagtctgggggaggcttggtgcagcctggggggtctctgagactctcctgtgtagcctctggattcaccttcaagagctatgccatggactgggtccgccaggctccagggaagggactcgagtggatcgcaggtatcaatagtgctggtagtccctcgtatgaagcctccgtgaagggccgattcaccatctccagagacaacgccgagaacacgctgtatctgcaattgaacagcctgaaaactgaggacacggccatgtattactgtacaaaatgtcgcgacttccgttcaccttattgtcgtccgggccagggcaccctggtcactgtctcatca

SEQ ID NO: 30 - protein, 118 aa, synthetic construct
  REGION 1..118: note = amino acid sequence of 1B-1A8 VHH
EVQLVESGGGLVQPGGSLRLSCVASGFTFKSYAMDWVRQAPGKGLEWIAGINSAGSPSYEASVKGRFTISRDNAENTLYLQLNSLKTEDTAMYYCTKCRDFRSPYCRPGQGTLVTVSS

SEQ ID NO: 31 - DNA, 372 bp, synthetic construct
  source 1..372: mol_type = other DNA
  gene 1..372: note = nucleotide sequence of 1B-1B2 VHH
gaggtgcagctggtggagtctgggggaggctcggtgcaggctggagggtctctgagactctcctgtacagcctctggattcacttttgatatgggctggtatcgccaggcgccaggagatgagtgcgagttggtctcaagtattagtagtgatggtaattcagactatttagactccgtgaagggccgattcaccatctcccaagacaacgccaagaatacggtgtatcttcaaatgaacagcctgaaacctgaggacacggccgtgtattactgtgcggcaaatggcgccggccatttggtgctccggccactgtgtggcagcaatgcagtggacgcatggggccaggggacactggtcactgtctcatca

SEQ ID NO: 32 - protein, 124 aa, synthetic construct
  REGION 1..124: note = amino acid sequence of 1B-1B2 VHH
EVQLVESGGGSVQAGGSLRLSCTASGFTFDMGWYRQAPGDECELVSSISSDGNSDYLDSVKGRFTISQDNAKNTVYLQMNSLKPEDTAVYYCAANGAGHLVLRPLCGSNAVDAWGQGTLVTVSS

SEQ ID NO: 33 - DNA, 378 bp, synthetic construct
  source 1..378: mol_type = other DNA
  gene 1..378: note = nucleotide sequence of 3B-1C7 VHH
caggtgcagctggtggagtctgggggagactcggtgcaggctggagggtctctgagactctcctgtatagcctctggattcacttttgatggcactactatgggctggtaccgccaggctccaggggatgagtgcgagttggtctcagatattagtagtgatggcaacacatactattcagactccgtgaagggccgattcactatctcccaaggcaacgccaagaacacggtgtatttgcaaatgaacagcctgacccctgaggacacggccgtatattactgtgcggctgctgagttcaggctcttgttgcgcccactctgtaggcaagatgactacggttattggggccaggggaccctggtcactgtctcatca

SEQ ID NO: 34 - protein, 126 aa, synthetic construct
  REGION 1..126: note = amino acid sequence of 3B-1C7 VHH
QVQLVESGGDSVQAGGSLRLSCIASGFTFDGTTMGWYRQAPGDECELVSDISSDGNTYYSDSVKGRFTISQGNAKNTVYLQMNSLTPEDTAVYYCAAAEFRLLLRPLCRQDDYGYWGQGTLVTVSS

SEQ ID NO: 35 - protein, 234 aa, synthetic construct
  REGION 1..234: note = amino acid sequence of HGFbeta
VVNGIPTRTNIGWMVSLRYRNKHICGGSLIKESWVLTARQCFPSRDLKDYEAWLGIHDVHGRGDEKCKQVLNVSQLVYGPEGSDLVLMKLARPAVLDDFVSTIDLPNYGCTIPEKTSCSVYGWGYTGLINYDGLLRVAHLYIMGNEKCSQHHRGKVTLNESEICAGAEKIGSGPCEGDYGGPLVCEQHKMRMVLGVIVPGRGCAIPNRPGIFVRVAYYAKWIHKIILTYKVPQS

SEQ ID NO: 36 - DNA, 1125 bp, synthetic construct
  source 1..1125: mol_type = other DNA
  gene 1..1125: note = nucleotide sequence of 1B-3B11-Fc
caggtgcagctggtggagtctgggggaggctcggtgcaggctggagggtctctgagactctcctgtgtagtctctggatacacctacagtagcgtggcctggttccgccaaactccagggaaggagcgcgagggggtcgctgttataaatcctggtggtgataacaccgactatacgtatgccgtgaagggccgattcaccatctcccgagacagcgccaagagcacggtgtttctgcaaatgaacaacctggaatctgaggacactgctatgtactactgtgcggcaggacggacgttcggtggcacatggatggatcggaataagtggaagtactggggccagggcaccctggtcactgtctcatcagaacctaagatccctcagcctcagcctaaaccacagccccagcctcagcctcaaccaaagcctcagcccaagcccgagcctgagtgcacctgtcctaagtgccctgctcctgaactgctgggaggcccttccgtgtttctgtttcctcccaagcctaaggacacactgatgatctctcggacccctgaagtgacctgcgtggtggtggatgtgtcccacgaggatcctgaggtcaagttcaactggtacgtggatggcgtggaagtgcacaatgctaaaaccaagcctagagaggaacagtacaactccacctacagagtggtgtccgtgctgaccgtgctgcaccaggattggctgaacggcaaagagtacaagtgcaaggtgtccaacaaggctctgcctgcccctatcgagaagaccatctccaaggccaagggacagcctcgggaacctcaggtgtacaccctgcctccttctagagacgagctgaccaagaaccaggtgtctctgacctgtctggtgaagggcttctaccctagcgacatcgccgtggagtgggagtccaatggacagcccgagaacaactacaagaccaccccacctgtgctggactccgacggctccttcttcctgtactccaagctgacagtggacaagtccagatggcagcagggcaacgtgttctcctgctccgtgatgcacgaggccctgcacaaccactacacccagaagtccctgtccctgtctcctggcaag

SEQ ID NO: 37 - protein, 375 aa, synthetic construct
  REGION 1..375: note = amino acid sequence of 1B-3B11-Fc
QVQLVESGGGSVQAGGSLRLSCVVSGYTYSSVAWFRQTPGKEREGVAVINPGGDNTDYTYAVKGRFTISRDSAKSTVFLQMNNLESEDTAMYYCAAGRTFGGTWMDRNKWKYWGQGTLVTVSSEPKIPQPQPKPQPQPQPQPKPQPKPEPECTCPKCPAPELLGGPSVFLFPPKPKDTLMISRTPEVTCVVVDVSHEDPEVKFNWYVDGVEVHNAKTKPREEQYNSTYRVVSVLTVLHQDWLNGKEYKCKVSNKALPAPIEKTISKAKGQPREPQVYTLPPSRDELTKNQVSLTCLVKGFYPSDIAVEWESNGQPENNYKTTPPVLDSDGSFFLYSKLTVDKSRWQQGNVFSCSVMHEALHNHYTQKSLSLSPGK

SEQ ID NO: 38 - DNA, 1149 bp, synthetic construct
  source 1..1149: mol_type = other DNA
  gene 1..1149: note = nucleotide sequence of 1B-1B6-Fc
caggtgcagctggtggagtctgggggagactcggtgcaggctggagggtctctgagactctcctgtgcagcctctgcacacgcctatagtagcggctgcatgggctggttccgccaggctccagggaagggccgcgagggggtcgcaactatttatactcgtaatgatttcacatactattccgactccgtgaagggccgattcaccatctcccgagacgacgccaagaacacggtgtatctgcaagtgaacagcctgaaagctgaggacactgccatgtactactgtgcggcaggttcacccttccggtacgctggtgcgtggaacgtctgcggcctgaaagaagaagactataactactggggccaggggaccctggtcactgtctcatcagaacctaagatccctcagcctcagcctaaaccacagccccagcctcagcctcaaccaaagcctcagcccaagcccgagcctgagtgcacctgtcctaagtgccctgctcctgaactgctgggaggcccttccgtgtttctgtttcctcccaagcctaaggacacactgatgatctctcggacccctgaagtgacctgcgtggtggtggatgtgtcccacgaggatcctgaggtcaagttcaactggtacgtggatggcgtggaagtgcacaatgctaaaaccaagcctagagaggaacagtacaactccacctacagagtggtgtccgtgctgaccgtgctgcaccaggattggctgaacggcaaagagtacaagtgcaaggtgtccaacaaggctctgcctgcccctatcgagaagaccatctccaaggccaagggacagcctcgggaacctcaggtgtacaccctgcctccttctagagacgagctgaccaagaaccaggtgtctctgacctgtctggtgaagggcttctaccctagcgacatcgccgtggagtgggagtccaatggacagcccgagaacaactacaagaccaccccacctgtgctggactccgacggctccttcttcctgtactccaagctgacagtggacaagtccagatggcagcagggcaacgtgttctcctgctccgtgatgcacgaggccctgcacaaccactacacccagaagtccctgtccctgtctcctggcaag

SEQ ID NO: 39 - protein, 383 aa, synthetic construct
  REGION 1..383: note = amino acid sequence of 1B-1B6-Fc
QVQLVESGGDSVQAGGSLRLSCAASAHAYSSGCMGWFRQAPGKGREGVATIYTRNDFTYYSDSVKGRFTISRDDAKNTVYLQVNSLKAEDTAMYYCAAGSPFRYAGAWNVCGLKEEDYNYWGQGTLVTVSSEPKIPQPQPKPQPQPQPQPKPQPKPEPECTCPKCPAPELLGGPSVFLFPPKPKDTLMISRTPEVTCVVVDVSHEDPEVKFNWYVDGVEVHNAKTKPREEQYNSTYRVVSVLTVLHQDWLNGKEYKCKVSNKALPAPIEKTISKAKGQPREPQVYTLPPSRDELTKNQVSLTCLVKGFYPSDIAVEWESNGQPENNYKTTPPVLDSDGSFFLYSKLTVDKSRWQQGNVFSCSVMHEALHNHYTQKSLSLSPGK

SEQ ID NO: 40 - DNA, 1140 bp, synthetic construct
  source 1..1140: mol_type = other DNA
  gene 1..1140: note = nucleotide sequence of 1B-1C7-Fc
caggtgcagctggtggagtctgggggaggcttggtgcagcctggggggtctctaagactctcctgtgcagcctctggatacagttacagtgctaactgcgtgggctggttctaccaggccccagggaaggagcgcgagggggtcgcagctatcaacactggtggtgaaacggcaacttatgccgacttcgtgaagggccgattcaccatctcccaagactacgccaagaacacggtgtatctgcaaatgaacagcctcaaatctgaggacactggcatgtactactgtgcggccgtagggacgaggaagtattgggacgagtgctccctttctcaacatgcgtataaaaactggggccagggcaccctggtcactgtctcatcagaacctaagatccctcagcctcagcctaaaccacagccccagcctcagcctcaaccaaagcctcagcccaagcccgagcctgagtgcacctgtcctaagtgccctgctcctgaactgctgggaggcccttccgtgtttctgtttcctcccaagcctaaggacacactgatgatctctcggacccctgaagtgacctgcgtggtggtggatgtgtcccacgaggatcctgaggtcaagttcaactggtacgtggatggcgtggaagtgcacaatgctaaaaccaagcctagagaggaacagtacaactccacctacagagtggtgtccgtgctgaccgtgctgcaccaggattggctgaacggcaaagagtacaagtgcaaggtgtccaacaaggctctgcctgcccctatcgagaagaccatctccaaggccaagggacagcctcgggaacctcaggtgtacaccctgcctccttctagagacgagctgaccaagaaccaggtgtctctgacctgtctggtgaagggcttctaccctagcgacatcgccgtggagtgggagtccaatggacagcccgagaacaactacaagaccaccccacctgtgctggactccgacggctccttcttcctgtactccaagctgacagtggacaagtccagatggcagcagggcaacgtgttctcctgctccgtgatgcacgaggccctgcacaaccactacacccagaagtccctgtccctgtctcctggcaag

SEQ ID NO: 41 - protein, 380 aa, synthetic construct
  REGION 1..380: note = amino acid sequence of 1B-1C7-Fc
QVQLVESGGGLVQPGGSLRLSCAASGYSYSANCVGWFYQAPGKEREGVAAINTGGETATYADFVKGRFTISQDYAKNTVYLQMNSLKSEDTGMYYCAAVGTRKYWDECSLSQHAYKNWGQGTLVTVSSEPKIPQPQPKPQPQPQPQPKPQPKPEPECTCPKCPAPELLGGPSVFLFPPKPKDTLMISRTPEVTCVVVDVSHEDPEVKFNWYVDGVEVHNAKTKPREEQYNSTYRVVSVLTVLHQDWLNGKEYKCKVSNKALPAPIEKTISKAKGQPREPQVYTLPPSRDELTKNQVSLTCLVKGFYPSDIAVEWESNGQPENNYKTTPPVLDSDGSFFLYSKLTVDKSRWQQGNVFSCSVMHEALHNHYTQKSLSLSPGK

SEQ ID NO: 42 - DNA, 1110 bp, synthetic construct
  source 1..1110: mol_type = other DNA
  gene 1..1110: note = nucleotide sequence of 1B-1A8-Fc
gaggtgcagctggtggagtctgggggaggcttggtgcagcctggggggtctctgagactctcctgtgtagcctctggattcaccttcaagagctatgccatggactgggtccgccaggctccagggaagggactcgagtggatcgcaggtatcaatagtgctggtagtccctcgtatgaagcctccgtgaagggccgattcaccatctccagagacaacgccgagaacacgctgtatctgcaattgaacagcctgaaaactgaggacacggccatgtattactgtacaaaatgtcgcgacttccgttcaccttattgtcgtccgggccagggcaccctggtcactgtctcatcagaacctaagatccctcagcctcagcctaaaccacagccccagcctcagcctcaaccaaagcctcagcccaagcccgagcctgagtgcacctgtcctaagtgccctgctcctgaactgctgggaggcccttccgtgtttctgtttcctcccaagcctaaggacacactgatgatctctcggacccctgaagtgacctgcgtggtggtggatgtgtcccacgaggatcctgaggtcaagttcaactggtacgtggatggcgtggaagtgcacaatgctaaaaccaagcctagagaggaacagtacaactccacctacagagtggtgtccgtgctgaccgtgctgcaccaggattggctgaacggcaaagagtacaagtgcaaggtgtccaacaaggctctgcctgcccctatcgagaagaccatctccaaggccaagggacagcctcgggaacctcaggtgtacaccctgcctccttctagagacgagctgaccaagaaccaggtgtctctgacctgtctggtgaagggcttctaccctagcgacatcgccgtggagtgggagtccaatggacagcccgagaacaactacaagaccaccccacctgtgctggactccgacggctccttcttcctgtactccaagctgacagtggacaagtccagatggcagcagggcaacgtgttctcctgctccgtgatgcacgaggccctgcacaaccactacacccagaagtccctgtccctgtctcctggcaag

SEQ ID NO: 43 - protein, 370 aa, synthetic construct
  REGION 1..370: note = amino acid sequence of 1B-1A8-Fc
EVQLVESGGGLVQPGGSLRLSCVASGFTFKSYAMDWVRQAPGKGLEWIAGINSAGSPSYEASVKGRFTISRDNAENTLYLQLNSLKTEDTAMYYCTKCRDFRSPYCRPGQGTLVTVSSEPKIPQPQPKPQPQPQPQPKPQPKPEPECTCPKCPAPELLGGPSVFLFPPKPKDTLMISRTPEVTCVVVDVSHEDPEVKFNWYVDGVEVHNAKTKPREEQYNSTYRVVSVLTVLHQDWLNGKEYKCKVSNKALPAPIEKTISKAKGQPREPQVYTLPPSRDELTKNQVSLTCLVKGFYPSDIAVEWESNGQPENNYKTTPPVLDSDGSFFLYSKLTVDKSRWQQGNVFSCSVMHEALHNHYTQKSLSLSPGK

SEQ ID NO: 44 - DNA, 1128 bp, synthetic construct
  source 1..1128: mol_type = other DNA
  gene 1..1128: note = nucleotide sequence of 1B-1B2-Fc
gaggtgcagctggtggagtctgggggaggctcggtgcaggctggagggtctctgagactctcctgtacagcctctggattcacttttgatatgggctggtatcgccaggcgccaggagatgagtgcgagttggtctcaagtattagtagtgatggtaattcagactatttagactccgtgaagggccgattcaccatctcccaagacaacgccaagaatacggtgtatcttcaaatgaacagcctgaaacctgaggacacggccgtgtattactgtgcggcaaatggcgccggccatttggtgctccggccactgtgtggcagcaatgcagtggacgcatggggccaggggacactggtcactgtctcatcagaacctaagatccctcagcctcagcctaaaccacagccccagcctcagcctcaaccaaagcctcagcccaagcccgagcctgagtgcacctgtcctaagtgccctgctcctgaactgctgggaggcccttccgtgtttctgtttcctcccaagcctaaggacacactgatgatctctcggacccctgaagtgacctgcgtggtggtggatgtgtcccacgaggatcctgaggtcaagttcaactggtacgtggatggcgtggaagtgcacaatgctaaaaccaagcctagagaggaacagtacaactccacctacagagtggtgtccgtgctgaccgtgctgcaccaggattggctgaacggcaaagagtacaagtgcaaggtgtccaacaaggctctgcctgcccctatcgagaagaccatctccaaggccaagggacagcctcgggaacctcaggtgtacaccctgcctccttctagagacgagctgaccaagaaccaggtgtctctgacctgtctggtgaagggcttctaccctagcgacatcgccgtggagtgggagtccaatggacagcccgagaacaactacaagaccaccccacctgtgctggactccgacggctccttcttcctgtactccaagctgacagtggacaagtccagatggcagcagggcaacgtgttctcctgctccgtgatgcacgaggccctgcacaaccactacacccagaagtccctgtccctgtctcctggcaag

SEQ ID NO: 45 - protein, 376 aa, synthetic construct
  REGION 1..376: note = amino acid sequence of 1B-1B2-Fc
EVQLVESGGGSVQAGGSLRLSCTASGFTFDMGWYRQAPGDECELVSSISSDGNSDYLDSVKGRFTISQDNAKNTVYLQMNSLKPEDTAVYYCAANGAGHLVLRPLCGSNAVDAWGQGTLVTVSSEPKIPQPQPKPQPQPQPQPKPQPKPEPECTCPKCPAPELLGGPSVFLFPPKPKDTLMISRTPEVTCVVVDVSHEDPEVKFNWYVDGVEVHNAKTKPREEQYNSTYRVVSVLTVLHQDWLNGKEYKCKVSNKALPAPIEKTISKAKGQPREPQVYTLPPSRDELTKNQVSLTCLVKGFYPSDIAVEWESNGQPENNYKTTPPVLDSDGSFFLYSKLTVDKSRWQQGNVFSCSVMHEALHNHYTQKSLSLSPGK

SEQ ID NO: 46 - DNA, 1134 bp, synthetic construct
  source 1..1134: mol_type = other DNA
  gene 1..1134: note = nucleotide sequence of 3B-1C7-Fc
caggtgcagctggtggagtctgggggagactcggtgcaggctggagggtctctgagactctcctgtatagcctctggattcacttttgatggcactactatgggctggtaccgccaggctccaggggatgagtgcgagttggtctcagatattagtagtgatggcaacacatactattcagactccgtgaagggccgattcactatctcccaaggcaacgccaagaacacggtgtatttgcaaatgaacagcctgacccctgaggacacggccgtatattactgtgcggctgctgagttcaggctcttgttgcgcccactctgtaggcaagatgactacggttattggggccaggggaccctggtcactgtctcatcagaacctaagatccctcagcctcagcctaaaccacagccccagcctcagcctcaaccaaagcctcagcccaagcccgagcctgagtgcacctgtcctaagtgccctgctcctgaactgctgggaggcccttccgtgtttctgtttcctcccaagcctaaggacacactgatgatctctcggacccctgaagtgacctgcgtggtggtggatgtgtcccacgaggatcctgaggtcaagttcaactggtacgtggatggcgtggaagtgcacaatgctaaaaccaagcctagagaggaacagtacaactccacctacagagtggtgtccgtgctgaccgtgctgcaccaggattggctgaacggcaaagagtacaagtgcaaggtgtccaacaaggctctgcctgcccctatcgagaagaccatctccaaggccaagggacagcctcgggaacctcaggtgtacaccctgcctccttctagagacgagctgaccaagaaccaggtgtctctgacctgtctggtgaagggcttctaccctagcgacatcgccgtggagtgggagtccaatggacagcccgagaacaactacaagaccaccccacctgtgctggactccgacggctccttcttcctgtactccaagctgacagtggacaagtccagatggcagcagggcaacgtgttctcctgctccgtgatgcacgaggccctgcacaaccactacacccagaagtccctgtccctgtctcctggcaag

SEQ ID NO: 47 - protein, 378 aa, synthetic construct
  REGION 1..378: note = amino acid sequence of 3B-1C7-Fc
QVQLVESGGDSVQAGGSLRLSCIASGFTFDGTTMGWYRQAPGDECELVSDISSDGNTYYSDSVKGRFTISQGNAKNTVYLQMNSLTPEDTAVYYCAAAEFRLLLRPLCRQDDYGYWGQGTLVTVSSEPKIPQPQPKPQPQPQPQPKPQPKPEPECTCPKCPAPELLGGPSVFLFPPKPKDTLMISRTPEVTCVVVDVSHEDPEVKFNWYVDGVEVHNAKTKPREEQYNSTYRVVSVLTVLHQDWLNGKEYKCKVSNKALPAPIEKTISKAKGQPREPQVYTLPPSRDELTKNQVSLTCLVKGFYPSDIAVEWESNGQPENNYKTTPPVLDSDGSFFLYSKLTVDKSRWQQGNVFSCSVMHEALHNHYTQKSLSLSPGK